European Patent Application EP 4 342 914 A1, published March 27, 2024. Title: ANTI-BCAM ANTIBODY OR ANTIGEN-BINDING FRAGMENT THEREOF. Applicant: Genome and Company. The sequence listing filed with the application follows.

SEQUENCE LISTING (24 sequences)

SEQ ID NO: 1 - protein, 120 aa, Artificial
  synthesized peptide
  misc_feature: 111a VH
QVTLKESGPGLVKPSGTLSLTCAVSGGSISSSNWWSWVRQPPGKGLEWIGEIYHSGSTNYNPSLKSRVTISVDKSKNQFSLKLSSVTAADTAVYYCARAYTVTTTYFDYWGQGTLVTVSS

SEQ ID NO: 2 - protein, 106 aa, Artificial
  synthesized peptide
  misc_feature: 111a VL
NIQMTQSPSTLSASVGDRVTITCRASQSMSTWLAWYQQKPGRAPKLLIYKASALETGVPSRFSGSGSGTQFTLTISSLQPDDFATYYCQQYDEFASFGQGTKVEIK

SEQ ID NO: 3 - protein, 125 aa, Artificial
  synthesized peptide
  misc_feature: 111b VH
EVQLVQSGAEVKKPGASVKVSCKASGYTFTSYYMHWVRQAPGQGLEWMGIINPSGGSTSYAQKFQGRVTMTRDTSTSTVYMELSSLRSEDTAVYYCARDGKGWDYYGSGSPLQYWGQGTLVTVSS

SEQ ID NO: 4 - protein, 110 aa, Artificial
  synthesized peptide
  misc_feature: 111b VL
LPVLTQPPSVSKGLRQTATLTCTGNSNNVGNQGAAWLQQHQGHPPKLLSYRNNDRPSGISERLSASRSGNTASLTITGLQPEDEADYYCSAWDSSLSAWVFGGGTKLTVL

SEQ ID NO: 5 - protein, 116 aa, Artificial
  synthesized peptide
  misc_feature: 111c VH
EVQLVQSGGGLVKPGGSLRLSCAASGFTFSDYYMSWIRQAPGKGLEWVSYTSSSGSTIYYADSVKGRFTISRDNAKNSLYLQMNSLRAEDTAVYYCARDITAFDIWGQGTMVTVSS

SEQ ID NO: 6 - protein, 110 aa, Artificial
  synthesized peptide
  misc_feature: 111c VL
LPVLTQPPSASGSPGQSVTISCTGTSSDVGGYNYVSWYQQHPGKAPKLMIYEVNKRPSGVPDRFSGSKSGNTASLTVSGLQAEDEADYYCCSYAGSNNYVFGTGTKVTVL

SEQ ID NO: 7 - protein, 11 aa, Artificial
  synthesized peptide
  misc_feature: 111a VH CDR1
GGSISSSNWWS

SEQ ID NO: 8 - protein, 11 aa, Artificial
  synthesized peptide
  misc_feature: 111a VL CDR1
RASQSMSTWLA

SEQ ID NO: 9 - protein, 10 aa, Artificial
  synthesized peptide
  misc_feature: 111b VH CDR1
GYTFTSYYMH

SEQ ID NO: 10 - protein, 13 aa, Artificial
  synthesized peptide
  misc_feature: 111b VL CDR1
TGNSNNVGNQGAA

SEQ ID NO: 11 - protein, 10 aa, Artificial
  synthesized peptide
  misc_feature: 111c VH CDR1
GFTFSDYYMS

SEQ ID NO: 12 - protein, 14 aa, Artificial
  synthesized peptide
  misc_feature: 111c VL CDR1
TGTSSDVGGYNYVS

SEQ ID NO: 13 - protein, 16 aa, Artificial
  synthesized peptide
  misc_feature: 111a VH CDR2
EIYHSGSTNYNPSLKS

SEQ ID NO: 14 - protein, 7 aa, Artificial
  synthesized peptide
  misc_feature: 111a VL CDR2
KASALET

SEQ ID NO: 15 - protein, 17 aa, Artificial
  synthesized peptide
  misc_feature: 111b VH CDR2
IINPSGGSTSYAQKFQG

SEQ ID NO: 16 - protein, 7 aa, Artificial
  synthesized peptide
  misc_feature: 111b VL CDR2
RNNDRPS

SEQ ID NO: 17 - protein, 17 aa, Artificial
  synthesized peptide
  misc_feature: 111c VH CDR2
YTSSSGSTIYYADSVKG

SEQ ID NO: 18 - protein, 7 aa, Artificial
  synthesized peptide
  misc_feature: 111c VL CDR2
EVNKRPS

SEQ ID NO: 19 - protein, 11 aa, Artificial
  synthesized peptide
  misc_feature: 111a VH CDR3
AYTVTTTYFDY

SEQ ID NO: 20 - protein, 8 aa, Artificial
  synthesized peptide
  misc_feature: 111a VL CDR3
QQYDEFAS

SEQ ID NO: 21 - protein, 16 aa, Artificial
  synthesized peptide
  misc_feature: 111b VH CDR3
DGKGWDYYGSGSPLQY

SEQ ID NO: 22 - protein, 11 aa, Artificial
  synthesized peptide
  misc_feature: 111b VL CDR3
SAWDSSLSAWV

SEQ ID NO: 23 - protein, 7 aa, Artificial
  synthesized peptide
  misc_feature: 111c VH CDR3
DITAFDI

SEQ ID NO: 24 - protein, 10 aa, Artificial
  synthesized peptide
  misc_feature: 111c VL CDR3
CSYAGSNNYV